European Patent Specification EP 3 297 670 B1, published July 2, 2025. Title: Molecular constructs with targeting and effector elements and their applications. Applicant: Immunwork Inc. The sequence listing filed with the application follows.

SEQUENCE LISTING (40 sequences)

SEQ ID NO: 1 - protein, 4 aa, Artificial Sequence
  filler sequence-1
GGGS

SEQ ID NO: 2 - protein, 4 aa, Artificial Sequence
  filler sequence-2
GSGS

SEQ ID NO: 3 - protein, 4 aa, Artificial Sequence
  filler sequence-3
GGSG

SEQ ID NO: 4 - protein, 5 aa, Artificial Sequence
  filler sequence-4
GSGGS

SEQ ID NO: 5 - protein, 5 aa, Artificial Sequence
  filler sequence-5
SGGSG

SEQ ID NO: 6 - protein, 5 aa, Artificial Sequence
  filler sequence-6
GGGGS

SEQ ID NO: 7 - protein, 6 aa, Artificial Sequence
  filler sequence-7
GGSGGS

SEQ ID NO: 8 - protein, 7 aa, Artificial Sequence
  filler sequence-8
GGSGGSG

SEQ ID NO: 9 - protein, 8 aa, Artificial Sequence
  filler sequence-9
SGSGGSGS

SEQ ID NO: 10 - protein, 9 aa, Artificial Sequence
  filler sequence-10
GSGGSGSGS

SEQ ID NO: 11 - protein, 10 aa, Artificial Sequence
  filler sequence-11
SGGSGGSGSG

SEQ ID NO: 12 - protein, 11 aa, Artificial Sequence
  filler sequence-12
GGSGGSGGSGS

SEQ ID NO: 13 - protein, 12 aa, Artificial Sequence
  filler sequence-13
SGGSGGSGSGGS

SEQ ID NO: 14 - protein, 13 aa, Artificial Sequence
  filler sequence-14
GGGGSGGSGGGGS

SEQ ID NO: 15 - protein, 14 aa, Artificial Sequence
  filler sequence-15
GGGSGSGSGSGGGS

SEQ ID NO: 16 - protein, 15 aa, Artificial Sequence
  filler sequence-16
SGSGGGGGSGGSGSG

SEQ ID NO: 17 - protein, 16 aa, Artificial Sequence
  MOD_RES 1: ACETYLATION
  polypeptide core-1
CGGSGGSGGSKGSGSK

SEQ ID NO: 18 - protein, 19 aa, Artificial Sequence
  MOD_RES 1: ACETYLATION
  polypeptitde core-2
CGGSGGSGGSKGSGSKGSK

SEQ ID NO: 19 - protein, 31 aa, Artificial Sequence
  MOD_RES 1: ACETYLATION
  polypeptide-3
CGSKGSKGSKGSKGSKGSKGSKGSKGSKGSK

SEQ ID NO: 20 - protein, 8 aa, Artificial Sequence
  hapten
WADWPGPP

SEQ ID NO: 21 - protein, 16 aa, Artificial Sequence
  MOD_RES 1: Xaa is homopropargylglycine
  MOD_RES 1: ACETYLATION
  polypeptide core-4
XGGSGGSGGSKGSGSK

SEQ ID NO: 22 - protein, 19 aa, Artificial Sequence
  MOD_RES 1: Xaa is homopropargylglycine
  MOD_RES 1: ACETYLATION
  polypeptide core-5
XGGSGGSGGSKGSGSKGSK

SEQ ID NO: 23 - protein, 19 aa, Artificial Sequence
  MOD_RES 1: Xaa is L-azidohomoalanine
  MOD_RES 1: ACETYLATION
  polypeptide core-6
XGGSGGSGGSKGSGSKGSK

SEQ ID NO: 24 - protein, 21 aa, Artificial Sequence
  MOD_RES 1: Xaa is homopropargylglycine
  MOD_RES 1: ACETYLATION
  polypeptide core-7
XGGSGGSGGSKGSGSKGSGSC

SEQ ID NO: 25 - protein, 7 aa, Artificial Sequence
  MOD_RES 1: ACETYLATION
  polypeptide core-8
  MOD_RES 2,4,6: Xaa is PEGylated amino acid with two EG units
CXKXKXK

SEQ ID NO: 26 - protein, 11 aa, Artificial Sequence
  MOD_RES 1: ACETYLATION
  polypeptide core-9
  MOD_RES 2,4,6,8,10: Xaa is PEGylated amino acid with six EG units
CXKXKXKXKXK

SEQ ID NO: 27 - protein, 16 aa, Artificial Sequence
  5xdrug
CGSKGSKGSKGSKGSK

SEQ ID NO: 28 - protein, 666 aa, Artificial Sequence
  human transferrin-1 receptor
LAGTESPVREEPGEDFPAARRLYWDDLKRKLSEKLDSTDFTSTIKLLNENSYVPREAGSQKDENLALYVENQFREFKLSKVWRDQHFVKIQVKDSAQNSVIIVDKNGRLVYLVENPGGYVAYSKAATVTGKLVHANFGTKKDFEDLYTPVNGSIVIVRAGKITFAEKVANAESLNAIGVLIYMDQTKFPIVNAELSFFGHAHLGTGDPYTPGFPSFNHTQFPPSRSSGLPNIPVQTISRAAAEKLFGNMEGDCPSDWKTDSTCRMVTSESKNVKLTVSNVLKEIKILNIFGVIKGFVEPDHYVVVGAQRDAWGPGAAKSGVGTALLLKLAQMFSDMVLKDGFQPSRSIIFASWSAGDFGSVGATEWLEGYLSSLHLKAFTYINLDKAVLGTSNFKVSASPLLYTLIEKTMQNVKHPVTGQFLYQDSNWASKVEKLTLDNAAFPFLAYSGIPAVSFCFCEDTDYPYLGTTMDTYKELIERIPELNKVARAAAEVAGQFVIKLTHDVELNLDYERYNSQLLSFVRDLNQYRADIKEMGLSLQWLYSARGDFFRATSRLTTDFGNAEKTDRFVMKKLNDRVMRVEYHFLSPYVSPKESPFRHVFWGSGSHTLPALLENLKLRKQNNGAFNETLFRNQLALATWTIQGAANALSGDVWDIDNEFHHHHHH

SEQ ID NO: 29 - protein, 192 aa, Artificial Sequence
  human CD32
QAAAPPKAVLKLEPPWINVLQEDSVTLTCQGARSPESDSIQWFHNGNLIPTHTQPSYRFKANNNDSGEYTCQTGQTSLSDPVHLTVLSEWLVLQTPHLEFQEGETIMLRCHSWKDKPLVKVTFFQNGKSQKFSRLDPTFSIPQANHSHSGDYHCTGNIGYTLFSSKPVTITVQVPSMGSSSPMGIIHHHHHH

SEQ ID NO: 30 - protein, 256 aa, Artificial Sequence
  scFv of anti-RSV mAb
DIQMTQSPSTLSASVGDRVTITCKCQLSVGYMHWYQQKPGKAPKLLIYDTSKLASGVPSRFSGSGSGTEFTLTISSLQPDDFATYYCFQGSGYPFTFGGGTKLEIKRGSTSGSGKPGSGEGSTKGQVTLRESGPALVKPTQTLTLTCTFSGFSLSTSGMSVGWIRQPPGKALEWLADIWWDDKKDYNPSLKSRLTISKDTSKNQVVLKVTNMDPADTATYYCARSMITNWYFDVWGAGTTVTVSSGGGGSGGGGSC

SEQ ID NO: 31 - protein, 257 aa, Artificial Sequence
  scFv of anti-endotoxin mAb
DIQMNQSPSSLSASLGDTISITCRASQNINIWLSWYQQKPGNVPKLLIYKASNLHTGVPSRFSGSGSGTDFTLIISSLQPEDIATYYCLQGQSYPRTFGGGTKLEIKRGSTSGSGKPGSGEGSTKGEVKLVESGGGLVQPGGSLSLSCAASGFTFSDYYMTWVRQAPGKAPEWLALIRNKRNGDTAEYSASVKGRFTISRDYSRSILHLQMNALRTEDSATYYCVRQGRGYTLDYWGQGTSVTVSSGGGGSGGGGSC

SEQ ID NO: 32 - protein, 255 aa, Artificial Sequence
  scFv of anti-CD32a mAb
AIQLTQSPSSLSASVGDRVTITCRASQGINSALAWYQQKPGKAPKLLIYDASSLESGVPSRFSGSGSGTDFTLTISSLQPEDFATYYCQQFNSYPHTFGQGTKLEIKRGSTSGSGKPGSGEGSTKGQVHLVESGGGVVQPGRSLRLSCAASGFTFSSYGMHWVRQAPGKGLEWVAVIWYDGSNYYYTDSVKGRFTISRDNSKNTLYLQMNSLRAEDTAVYYCARDLGAAASDYWGQGTLVTVSSGGGGSGGGGSC

SEQ ID NO: 33 - protein, 251 aa, Artificial Sequence
  scFv of anti-transferrin-1 receptor mAb
DIVITQSPSSLSASLGDTILITCHASQNINVWLSWFQQKPGNAPKLLIYKASNLHTGVPSRFSGSGSGTGFTLTISSLQPEDIATYYCQQGQSYPWTFGGGTKLEIKRGSTSGSGKPGSGEGSTKGQVQLQQPGAALVRPGASMRLSCKASGYSFTTYWMNWVKQRPGQGLELIGMIHPSDSEVRLNQKFKDKATLTVDTSSSTAYMQLNSPTSEDSAVYYCARFGLDYWGQGTTLTVSSGGGGSGGGGSC

SEQ ID NO: 34 - protein, 262 aa, Artificial Sequence
  scFv of anti-beta-amyloid Bapineuzumab mAb
DVVMTQSPLSLPVTPGEPASISCKSSQSLLDSDGKTYLNWLLQKPGQSPQRLIYLVSKLDSGVPDRFSGSGSGTDFTLKISRVEAEDVGVYYCWQGTHFPRTFGQGTKVEIKRGSTSGSGKPGSGEGSTKGEVQLLESGGGLVQPGGSLRLSCAASGFTFSNYGMSWVRQAPGKGLEWVASIRSGGGRTYYSDNVKGRFTISRDNSKNTLYLQMNSLRAEDTAVYYCVRYDHYSGSSDYWGQGTLVTVSSAGGGGSGGGGSC

SEQ ID NO: 35 - protein, 239 aa, Artificial Sequence
  B6 scFv of anti-human TfR derived from phage display
DIQMTQSPSSLSASVGDRVTITCRASQDVDSDVAWYQQKPGKAPKLLISYSGYLYSGVPSRFSGSGSGTDFTLTISSLQPEDFATYYCQQSWGFPLTFGQGTKVEIKRGGGGSIEGRSGGGGSEVQLVESGGGLVQPGGSLRLSCAASGFTIGNSSIHWVRQAPGKGLEWVASIWPFGGSTYYADSVKGRFTISADTSKNTAYLQMNSLRAEDTAVYYCARWSYGFDYWGQGTLVTVSS

SEQ ID NO: 36 - protein, 243 aa, Artificial Sequence
  scFv of anti-human CD32 derived from phage display
DIQMTQSPSSLSASVGDRVTITCRASQDVNNGVAWYQQKPGKAPKLLIFGTSGLYSGVPSRFSGSGSGTDFTLTISSLQPEDFATYYCQQGFGGPMTFGQGTKVEIKRGGSSRSSSSGGGGSGGGGEVQLVESGGGLVQPGGSLRLSCAASGFTINNGGIHWVRQAPGKGLEWVAGIWPFGGFTSYADSVKGRFTISADTSKNTAYLQMNSLRAEDTAVYYCARSWFSWSDYWGQGTLVTVSS

SEQ ID NO: 37 - protein, 737 aa, Artificial Sequence
  (anti-RSV scfv)-IgG1.Fc-(anti-CD32 scFv)
DIQMTQSPSTLSASVGDRVTITCKCQLSVGYMHWYQQKPGKAPKLLIYDTSKLASGVPSRFSGSGSGTEFTLTISSLQPDDFATYYCFQGSGYPFTFGGGTKLEIKRGSTSGSGKPGSGEGSTKGQVTLRESGPALVKPTQTLTLTCTFSGFSLSTSGMSVGWIRQPPGKALEWLADIWWDDKKDYNPSLKSRLTISKDTSKNQVVLKVTNMDPADTATYYCARSMITNWYFDVWGAGTTVTVSSASGGSGGGGSGGGGSPAPELLGGPSVFLFPPKPKDTLMISRTPEVTCVVVDVSHEDPEVKFNWYVDGVEVHNAKTKPREEQYNSTYRVVSVLTVLHQDWLNGKDYKCKVSNKALPAPIEKTISKAKGQPREPQVYTLPPSRDELTRNQVSLTCLVKGFYPSDIAVEWESNGQPENNYKTTPPVLDSDGSFFLYSKLTVDKSRWQQGNVFSCSVMHEALHNHYTQKSLSLSPGKGGGGSGGGGSGGGGSAIQLTQSPSSLSASVGDRVTITCRASQGINSALAWYQQKPGKAPKLLIYDASSLESGVPSRFSGSGSGTDFTLTISSLQPEDFATYYCQQFNSYPHTFGQGTKLEIKRGSTSGSGKPGSGEGSTKGQVHLVESGGGVVQPGRSLRLSCAASGFTFSSYGMHWVRQAPGKGLEWVAVIWYDGSNYYYTDSVKGRFTISRDNSKNTLYLQMNSLRAEDTAVYYCARDLGAAASDYWGQGTLVTVSS

SEQ ID NO: 38 - protein, 738 aa, Artificial Sequence
  (anti-endotoxin scfv)-IgG1.Fc-(anti-CD32 scFv)
DIQMNQSPSSLSASLGDTISITCRASQNINIWLSWYQQKPGNVPKLLIYKASNLHTGVPSRFSGSGSGTDFTLIISSLQPEDIATYYCLQGQSYPRTFGGGTKLEIKRGSTSGSGKPGSGEGSTKGEVKLVESGGGLVQPGGSLSLSCAASGFTFSDYYMTWVRQAPGKAPEWLALIRNKRNGDTAEYSASVKGRFTISRDYSRSILHLQMNALRTEDSATYYCVRQGRGYTLDYWGQGTSVTVSSASGGSGGGGSGGGGSPAPELLGGPSVFLFPPKPKDTLMISRTPEVTCVVVDVSHEDPEVKFNWYVDGVEVHNAKTKPREEQYNSTYRVVSVLTVLHQDWLNGKDYKCKVSNKALPAPIEKTISKAKGQPREPQVYTLPPSRDELTRNQVSLTCLVKGFYPSDIAVEWESNGQPENNYKTTPPVLDSDGSFFLYSKLTVDKSRWQQGNVFSCSVMHEALHNHYTQKSLSLSPGKGGGGSGGGGSGGGGSAIQLTQSPSSLSASVGDRVTITCRASQGINSALAWYQQKPGKAPKLLIYDASSLESGVPSRFSGSGSGTDFTLTISSLQPEDFATYYCQQFNSYPHTFGQGTKLEIKRGSTSGSGKPGSGEGSTKGQVHLVESGGGVVQPGRSLRLSCAASGFTFSSYGMHWVRQAPGKGLEWVAVIWYDGSNYYYTDSVKGRFTISRDNSKNTLYLQMNSLRAEDTAVYYCARDLGAAASDYWGQGTLVTVSS

SEQ ID NO: 39 - protein, 658 aa, Artificial Sequence
  (IFN-beta)Avonex-IgG4.Fc-(anti-TfR scFv)
MSYNLLGFLQRSSNFQCQKLLWQLNGRLEYCLKDRMNFDIPEEIKQLQQFQKEDAALTIYEMLQNIFAIFRQDSSSTGWNETIVENLLANVYHQINHLKTVLEEKLEKEDFTRGKLMSSLHLKRYYGRILHYLKAKEYSHCAWTIVRVEILRNFYFINRLTGYLRNGGGGSGGGASGGSPPCPSCPAPEFLGGPSVFLFPPKPKDTLMISRTPEVTCVVVDVSQEDPEVQFNWYVDGVEVHNAKTKPREEQFNSTYRVVSVLTVLHQDWLNGKEYKCKVSNKGLPSSIEKTISKAKGQPREPQVYTLPPSQEEMTKNQVSLTCLVKGFYPSDIAVEWESNGQPENNYKTTPPVLDSDGSFFLYSRLTVDKSRWQEGNVFSCSVMHEALHNHYTQKSLSLSLGKGGGGSGGGGSGGGGSDIVITQSPSSLSASLGDTILITCHASQNINVWLSWFQQKPGNAPKLLIYKASNLHTGVPSRFSGSGSGTGFTLTISSLQPEDIATYYCQQGQSYPWTFGGGTKLEIKRGSTSGSGKPGSGEGSTKGQVQLQQPGAALVRPGASMRLSCKASGYSFTTYWMNWVKQRPGQGLELIGMIHPSDSEVRLNQKFKDKATLTVDTSSSTAYMQLNSPTSEDSAVYYCARFGLDYWGQGTTLTVSS

SEQ ID NO: 40 - protein, 738 aa, Artificial Sequence
  (anti-integrin a4 scfv)--IgG4.Fc-(anti-TfR scFv)
SIVMTQTPKFLLVSAGDRVTITCKASQSVTNDVAWYQQKPGQSPKLLIYYASNRYTGVPDRFTGSGYGTDFTFTISTVQAEDLAVYFCQQDYSSPYTFGGGTKLEIKRGSTSGSGKPGSGEGSTKGVKLQQSGAELVKPGASVKLFCTASGFNIKDTYMHWVKQRPQQGLEWIGRIDPASGDTKYDPKFQVKATITADTSSNTAWLQLSSLTSEDTAVYYCADGMWVSTGYALDFWGQGTTVTVSSGGGGSGGGASGGSPPCPSCPAPEFLGGPSVFLFPPKPKDTLMISRTPEVTCVVVDVSQEDPEVQFNWYVDGVEVHNAKTKPREEQFNSTYRVVSVLTVLHQDWLNGKEYKCKVSNKGLPSSIEKTISKAKGQPREPQVYTLPPSQEEMTKNQVSLTCLVKGFYPSDIAVEWESNGQPENNYKTTPPVLDSDGSFFLYSRLTVDKSRWQEGNVFSCSVMHEALHNHYTQKSLSLSLGKGGGGSGGGGSGGGGSDIVITQSPSSLSASLGDTILITCHASQNINVWLSWFQQKPGNAPKLLIYKASNLHTGVPSRFSGSGSGTGFTLTISSLQPEDIATYYCQQGQSYPWTFGGGTKLEIKRGSTSGSGKPGSGEGSTKGQVQLQQPGAALVRPGASMRLSCKASGYSFTTYWMNWVKQRPGQGLELIGMIHPSDSEVRLNQKFKDKATLTVDTSSSTAYMQLNSPTSEDSAVYYCARFGLDYWGQGTTLTVSS